European Patent Application EP 4 585 226 A1, published July 16, 2025. Title: Agent for treating infectious disease by corona virus. Applicant: Innate Cell Therapy Inc. Application WO. The sequence listing filed with the application follows.

SEQUENCE LISTING (12 sequences)

SEQ ID NO: 1 - DNA, 1638 bp, Homo sapiens
  source 1..1638: mol_type = other DNA
atgcttttgagccagaatgccttcatcttcagatcacttaatttggttctcatggtgtatatcagcctcgtgtttggtatttcatatgattcgcctgattacacagatgaatcttgcactttcaagatatcattgcgaaatttccggtccatcttatcatgggaattaaaaaaccactccattgtaccaactcactatacattgctgtatacaatcatgagtaaaccagaagatttgaaggtggttaagaactgtgcaaataccacaagatcattttgtgacctcacagatgagtggagaagcacacacgaggcctatgtcaccgtcctagaaggattcagcgggaacacaacgttgttcagttgctcacacaatttctggctggccatagacatgtcttttgaaccaccagagtttgagattgttggttttaccaaccacattaatgtgatggtgaaatttccatctattgttgaggaagaattacagtttgatttatctctcgtcattgaagaacagtcagagggaattgttaagaagcataaacccgaaataaaaggaaacatgagtggaaatttcacctatatcattgacaagttaattccaaacacgaactactgtgtatctgtttatttagagcacagtgatgagcaagcagtaataaagtctcccttaaaatgcaccctccttccacctggccaggaatcagcattgggaatggtaccacctcccgaaaatgtcagaatgaattctgttaatttcaagaacattctacagtgggagtcacctgcttttgccaaagggaacctgactttcacagctcagtacctaagttataggatattccaagataaatgcatgaatactaccttgacggaatgtgatttctcaagtctttccaagtatggtgaccacaccttgagagtcagggctgaatttgcagatgagcattcagactgggtaaacatcaccttctgtcctgtggatgacaccattattggaccccctggaatgcaagtagaagtacttgctgattctttacatatgcgtttcttagcccctaaaattgagaatgaatacgaaacttggactatgaagaatgtgtataactcatggacttataatgtgcaatactggaaaaacggtactgatgaaaagtttcaaattactccccagtatgactttgaggtcctcagaaacctggagccatggacaacttattgtgttcaagttcgagggtttcttcctgatcggaacaaagctggggaatggagtgagcctgtctgtgagcaaacaacccatgacgaaacggtcccctcctggatggtggccgtcatcctcatggcctcggtcttcatggtctgcctggcactcctcggctgcttcgccttgctgtggtgcgtttacaagaagacaaagtacgccttctcccctaggaattctcttccacagcacctgaaagagtttttgggccatcctcatcataacacacttctgtttttctcctttccattgtcggatgagaatgatgtttttgacaagctaagtgtcattgcagaagactctgagagcggcaagcagaatcctggtgacagctgcagcctcgggaccccgcctgggcaggggccccaaagctag

SEQ ID NO: 2 - protein, 545 aa, Homo sapiens
MLLSQNAFIFRSLNLVLMVYISLVFGISYDSPDYTDESCTFKISLRNFRSILSWELKNHSIVPTHYTLLYTIMSKPEDLKVVKNCANTTRSFCDLTDEWRSTHEAYVTVLEGFSGNTTLFSCSHNFWLAIDMSFEPPEFEIVGFTNHINVMVKFPSIVEEELQFDLSLVIEEQSEGIVKKHKPEIKGNMSGNFTYIIDKLIPNTNYCVSVYLEHSDEQAVIKSPLKCTLLPPGQESALGMVPPPENVRMNSVNFKNILQWESPAFAKGNLTFTAQYLSYRIFQDKCMNTTLTECDFSSLSKYGDHTLRVRAEFADEHSDWVNITFCPVDDTIIGPPGMQVEVLADSLHMRFLAPKIENEYETWTMKNVYNSWTYNVQYWKNGTDEKFQITPQYDFEVLRNLEPWTTYCVQVRGFLPDRNKAGEWSEPVCEQTTHDETVPSWMVAVILMASVFMVCLALLGCFALLWCVYKKTKYAFSPRNSLPQHLKEFLGHPHHNTLLFFSFPLSDENDVFDKLSVIAEDSESGKQNPGDSCSLGTPPGQGPQS

SEQ ID NO: 3 - DNA, 1638 bp, Homo sapiens
  source 1..1638: mol_type = other DNA
atgcttttgagccagaatgccttcatcttcagatcacttaatttggttctcatggtgtatatcagcctcgtgtttggtatttcatatgattcgcctgattacacagatgaatcttgcactttcaagatatcattgcgaaatttccggtccatcttatcatgggaattaaaaaaccactccattgtaccaactcactatacattgctgtatacaatcatgagtaaaccagaagatttgaaggtggttaagaactgtgcaaataccacaagatcattttgtgacctcacagatgagtggagaagcacacacgaggcctatgtcaccgtcctagaaggattcagcgggaacacaacgttgttcagttgctcacacaatttctggctggccatagacatgtcttttgaaccaccagagtttgagattgttggttttaccaaccacattaatgtgatggtgaaatttccatctattgttgaggaagaattacagtttgatttatctctcgtcattgaagaacagtcagagggaattgttaagaagcataaacccgaaataaaaggaaacatgagtggaaatttcacctatatcattgacaagttaattccaaacacgaactactgtgtatctgtttatttagagcacagtgatgagcaagcagtaataaagtctcccttaaaatgcaccctccttccacctggccaggaatcagcattgggaatggtaccacctcccgaaaatgtcagaatgaattctgttaatttcaagaacattctacagtgggagtcacctgcttttgccgaagggaacctgactttcacagctcagtacctaagttataggatattccaagataaatgcatgaatactaccttgacggaatgtgatttctcaagtctttccaagtatggtgaccacaccttgagagtcagggctgaatttgcagatgagcattcagactgggtaaacatcaccttctgtcctgtggatgacaccattattggaccccctggaatgcaagtagaagtacttgctgattctttacatatgcgtttcttagcccctaaaattgagaatgaatacgaaacttggactatgaagaatgtgtataactcatggacttataatgtgcaatactggaaaaacggtactgatgaaaagtttcaaattactccccagtatgactttgaggtcctcagaaacctggagccatggacaacttattgtgttcaagttcgagggtttcttcctgatcggaacaaagctggggaatggagtgagcctgtctgtgagcaaacaacccatgacgaaacggtcccctcctggatggtggccgtcatcctcatggcctcggtcttcatggtctgcctggcactcctcggctgcttcgccttgctgtggtgcgtttacaagaagacaaagtacgccttctcccctaggaattctcttccacagcacctgaaagagtttttgggccatcctcatcataacacacttctgtttttctcctttccattgtcggatgagaatgatgtttttgacaagctaagtgtcattgcagaagactctgagagcggcaagcagaatcctggtgacagctgcagcctcgggaccccgcctgggcaggggccccaaagctag

SEQ ID NO: 4 - protein, 545 aa, Homo sapiens
MLLSQNAFIFRSLNLVLMVYISLVFGISYDSPDYTDESCTFKISLRNFRSILSWELKNHSIVPTHYTLLYTIMSKPEDLKVVKNCANTTRSFCDLTDEWRSTHEAYVTVLEGFSGNTTLFSCSHNFWLAIDMSFEPPEFEIVGFTNHINVMVKFPSIVEEELQFDLSLVIEEQSEGIVKKHKPEIKGNMSGNFTYIIDKLIPNTNYCVSVYLEHSDEQAVIKSPLKCTLLPPGQESALGMVPPPENVRMNSVNFKNILQWESPAFAEGNLTFTAQYLSYRIFQDKCMNTTLTECDFSSLSKYGDHTLRVRAEFADEHSDWVNITFCPVDDTIIGPPGMQVEVLADSLHMRFLAPKIENEYETWTMKNVYNSWTYNVQYWKNGTDEKFQITPQYDFEVLRNLEPWTTYCVQVRGFLPDRNKAGEWSEPVCEQTTHDETVPSWMVAVILMASVFMVCLALLGCFALLWCVYKKTKYAFSPRNSLPQHLKEFLGHPHHNTLLFFSFPLSDENDVFDKLSVIAEDSESGKQNPGDSCSLGTPPGQGPQS

SEQ ID NO: 5 - DNA, 27 bp, Artificial Sequence
  source 1..27: mol_type = other DNA
ggatccatgcttttgagccagaatgcc

SEQ ID NO: 6 - DNA, 24 bp, Artificial Sequence
  source 1..24: mol_type = other DNA
ctcgagctagctttggggcccctg

SEQ ID NO: 7 - DNA, 23 bp, Artificial Sequence
  source 1..23: mol_type = other DNA
aacatgagtggaaatttcaccta

SEQ ID NO: 8 - DNA, 21 bp, Artificial Sequence
  source 1..21: mol_type = other DNA
ggtaccattcccaatgctgat

SEQ ID NO: 9 - DNA, 23 bp, Artificial Sequence
  source 1..23: mol_type = other DNA
tgacaagttaattccaaacacga

SEQ ID NO: 10 - DNA, 22 bp, Artificial Sequence
  source 1..22: mol_type = other DNA
gaggcatagtttcactctgttg

SEQ ID NO: 11 - DNA, 20 bp, Artificial Sequence
  source 1..20: mol_type = other DNA
ctggacacagtggctcatac

SEQ ID NO: 12 - DNA, 21 bp, Artificial Sequence
  source 1..21: mol_type = other DNA
cagtggctcatacctgtaacc